European Patent Application EP 4 249 500 A2, published September 27, 2023. Title: Peptide entities with antimicrobial action against multidrug resistant pathogens. Applicant: Centro de Investigación y Desarrollo de Medicamentos CIDEM. The sequence listing filed with the application follows.

SEQUENCE LISTING (3 sequences)

SEQ ID NO: 1 - protein, 27 aa, artificial sequence
  Synthetic Construct
  PEPTIDE (1)..(27): Xaa= Arg or Lys in their L or D conformation, with at least four Arg residues
  DISULFID (2)..(23)
  MISC_FEATURE (7)..(7): Xaa=Arg, Lys
  MISC_FEATURE (13)..(13): Xaa=Arg, Lys
  MISC_FEATURE (15)..(15): Xaa=Arg, Lys
  MISC_FEATURE (21)..(21): Xaa=Arg, Lys
  MISC_FEATURE (24)..(24): Xaa=Arg, Lys
  MISC_FEATURE (25)..(25): Xaa=Arg, Lys
  MISC_FEATURE (25)..(25): Xaa= Arg; Lys
  MOD_RES (27)..(27): AMIDATION
YCPYGNXLNYWSXAXGHIGTXSCXXSY

SEQ ID NO: 2 - protein, 28 aa, artificial sequence
  Synthetic Construct
  PEPTIDE (1)..(28): Xaa= Arg or Lys in their L or D conformation, with at least four Arg residues
  DISULFID (5)..(22)
  MISC_FEATURE (6)..(6)
  MISC_FEATURE (9)..(9)
  MISC_FEATURE (13)..(13): Xaa= Arg; Lys
  MISC_FEATURE (20)..(20): Xaa= Arg; Lys
  MISC_FEATURE (24)..(24): Xaa= Arg; Lys
  MISC_FEATURE (25)..(25): Xaa= Arg; Lys
  MOD_RES (28)..(28): AMIDATION
YSTSCXYFXLDYXSFSVGTXSCVXXGIY

SEQ ID NO: 3 - protein, 28 aa, artificial sequence
  synthetic variant for hybrid peptide
  PEPTIDE (1)..(28): Xaa= Arg or Lys in their L or D conformation, with at least four Arg residues
  DISULFID (5)..(22)
  MISC_FEATURE (6)..(6): Xaa= Arg; Lys
  MISC_FEATURE (9)..(9): Xaa= Arg; Lys
  MISC_FEATURE (15)..(15): Xaa= Arg; Lys
  MISC_FEATURE (17)..(17): Xaa= Arg; Lys
  MISC_FEATURE (24)..(24): Xaa= Arg; Lys
  MISC_FEATURE (25)..(25): Xaa= Arg; Lys
  MOD_RES (28)..(28): AMIDATION
YSTSCXYFXLNHWSXAXGHISCVXXGIY